European Patent Application EP 4 134 368 A1, published February 15, 2023. Title: TRIAZOLOPYRIMIDINE COMPOUNDS AND THEIR USE IN TREATING CANCER. Applicant: AstraZeneca AB. The sequence listing filed with the application follows.

SEQUENCE LISTING (1 sequence)

SEQ ID NO: 1 - DNA, 1398 bp, Artificial Sequence
  DNA encoding human MCT4
atgggaggggccgtggtggacgagggccccacaggcgtcaaggcccctgacggcggctggggctgggccgtgctcttcggctgtttcgtcatcactggcttctcctacgccttccccaaggccgtcagtgtcttcttcaaggagctcatacaggagtttgggatcggctacagcgacacagcctggatctcctccatcctgctggccatgctctacgggacaggtccgctctgcagtgtgtgcgtgaaccgctttggctgccggcccgtcatgcttgtggggggtctctttgcgtcgctgggcatggtggctgcgtccttttgccggagcatcatccaggtctacctcaccactggggtcatcacggggttgggtttggcactcaacttccagccctcgctcatcatgctgaaccgctacttcagcaagcggcgccccatggccaacgggctggcggcagcaggtagccctgtcttcctgtgtgccctgagcccgctggggcagctgctgcaggaccgctacggctggcggggcggcttcctcatcctgggcggcctgctgctcaactgctgcgtgtgtgccgcactcatgaggcccctggtggtcacggcccagccgggctcggggccgccgcgaccctcccggcgcctgctagacctgagcgtcttccgggaccgcggctttgtgctttacgccgtggccgcctcggtcatggtgctggggctcttcgtcccgcccgtgttcgtggtgagctacgccaaggacctgggcgtgcccgacaccaaggccgccttcctgctcaccatcctgggcttcattgacatcttcgcgcggccggccgcgggcttcgtggcggggcttgggaaggtgcggccctactccgtctacctcttcagcttctccatgttcttcaacggcctcgcggacctggcgggctctacggcgggcgactacggcggcctcgtggtcttctgcatcttctttggcatctcctacggcatggtgggggccctgcagttcgaggtgctcatggccatcgtgggcacccacaagttctccagtgccattggcctggtgctgctgatggaggcggtggccgtgctcgtcgggcccccttcgggaggcaaactcctggatgcgacccacgtctacatgtacgtgttcatcctggcgggggccgaggtgctcacctcctccctgattttgctgctgggcaacttcttctgcattaggaagaagcccaaagagccacagcctgaggtggcggccgcggaggaggagaagctccacaagcctcctgcagactcgggggtggacttgcgggaggtggagcatttcctgaaggctgagcctgagaaaaacggggaggtggttcacaccccggaaacaagtgtctga